European Patent Application EP 4 428 144 A1, published September 11, 2024. Title: Peptide Having Physiological Activity and Use Thereof. Applicant: CAREGEN CO., LTD. The sequence listing filed with the application follows.

SEQUENCE LISTING (19 sequences)

SEQ ID NO: 1 - protein, 10 aa, synthetic construct
  REGION 1..10: note = peptide having cartilage regeneration activity
ACDWGLWWLC

SEQ ID NO: 2 - DNA, 23 bp, synthetic construct
  misc_feature 1..23: note = forward primer for hCOL2A1 gene
  source 1..23: mol_type = other DNA
ctatctggacgaagcagctggca

SEQ ID NO: 3 - DNA, 22 bp, synthetic construct
  misc_feature 1..22: note = reverse primer for hCOL2A1 gene
  source 1..22: mol_type = other DNA
atgggtgcaatgtcaatgatgg

SEQ ID NO: 4 - DNA, 20 bp, synthetic construct
  misc_feature 1..20: note = forward primer for hACAN gene
  source 1..20: mol_type = other DNA
gcaggctatgagcagtgtga

SEQ ID NO: 5 - DNA, 20 bp, synthetic construct
  misc_feature 1..20: note = reverse primer for hACAN gene
  source 1..20: mol_type = other DNA
gcatacctcggaagcagaag

SEQ ID NO: 6 - DNA, 20 bp, synthetic construct
  misc_feature 1..20: note = forward primer for hPCP gene
  source 1..20: mol_type = other DNA
tgagtcctcaagcctcctgt

SEQ ID NO: 7 - DNA, 20 bp, synthetic construct
  misc_feature 1..20: note = reverse primer for hPCP gene
  source 1..20: mol_type = other DNA
gtgccagatcatcaccacac

SEQ ID NO: 8 - DNA, 20 bp, synthetic construct
  misc_feature 1..20: note = forward primer for GAPDH gene
  source 1..20: mol_type = other DNA
accacagtccatgccatcac

SEQ ID NO: 9 - DNA, 20 bp, synthetic construct
  misc_feature 1..20: note = reverse primer for GAPDH gene
  source 1..20: mol_type = other DNA
tccaccaccctgttgctgta

SEQ ID NO: 10 - DNA, 20 bp, synthetic construct
  misc_feature 1..20: note = forward primer for hCOMP gene
  source 1..20: mol_type = other DNA
aactcagggcaggaggatgt

SEQ ID NO: 11 - DNA, 20 bp, synthetic construct
  misc_feature 1..20: note = reverse primer for hCOMP gene
  source 1..20: mol_type = other DNA
tgtccttttggtcgtcgttc

SEQ ID NO: 12 - DNA, 20 bp, synthetic construct
  misc_feature 1..20: note = forward primer for hCOL11A gene
  source 1..20: mol_type = other DNA
ccagcccgaacttgtaaaga

SEQ ID NO: 13 - DNA, 20 bp, synthetic construct
  misc_feature 1..20: note = reverse primer for hCOL11A gene
  source 1..20: mol_type = other DNA
tggacgcacaaccatcatac

SEQ ID NO: 14 - DNA, 20 bp, synthetic construct
  misc_feature 1..20: note = forward primer for TNF-alpha gene
  source 1..20: mol_type = other DNA
cgtcagccgatttgctatct

SEQ ID NO: 15 - DNA, 20 bp, synthetic construct
  misc_feature 1..20: note = reverse primer for TNF-alpha gene
  source 1..20: mol_type = other DNA
cggactccgcaaagtctaag

SEQ ID NO: 16 - DNA, 20 bp, synthetic construct
  misc_feature 1..20: note = forward primer for IL-1beta gene
  source 1..20: mol_type = other DNA
caaggagaaccaagcaacga

SEQ ID NO: 17 - DNA, 20 bp, synthetic construct
  misc_feature 1..20: note = reverse primer for IL-1beta gene
  source 1..20: mol_type = other DNA
ttggccgaggactaaggagt

SEQ ID NO: 18 - DNA, 20 bp, synthetic construct
  misc_feature 1..20: note = forward primer for Cox2 gene
  source 1..20: mol_type = other DNA
tgagtggtagccagcaaagc

SEQ ID NO: 19 - DNA, 20 bp, synthetic construct
  misc_feature 1..20: note = reverse primer for Cox2 gene
  source 1..20: mol_type = other DNA
ctgcagtccaggttcaatgg